European Patent Specification EP 4 536 267 B1, published April 29, 2026. Title: Hémoglobine d'Annélides pour son utilisation dans le traitement de la maladie de Fuchs. Applicant: Hemarina et al. The sequence listing filed with the application follows.

SEQUENCE LISTING (22 sequences)

SEQ ID NO: 1 - DNA, 20 bp, synthetic construct
  misc_feature 1..20: note = amorce forward BAG3
  source 1..20: mol_type = other DNA
ggagatcaagatcgacccgc

SEQ ID NO: 2 - DNA, 21 bp, synthetic construct
  misc_feature 1..21: note = amorce reverse BAG3
  source 1..21: mol_type = other DNA
agaggatggagtctccttggg

SEQ ID NO: 3 - DNA, 20 bp, synthetic construct
  misc_feature 1..20: note = amorce forward B2M
  source 1..20: mol_type = other DNA
actgaattcacccccactga

SEQ ID NO: 4 - DNA, 20 bp, synthetic construct
  misc_feature 1..20: note = amorce reverse B2M
  source 1..20: mol_type = other DNA
cctccatgatgctgcttaca

SEQ ID NO: 5 - DNA, 23 bp, synthetic construct
  misc_feature 1..23: note = amorce forward CD166
  source 1..23: mol_type = other DNA
ccccagaggaatttttgttttac

SEQ ID NO: 6 - DNA, 23 bp, synthetic construct
  misc_feature 1..23: note = amorce reverse CD166
  source 1..23: mol_type = other DNA
agcctgatgttatctttcatcca

SEQ ID NO: 7 - DNA, 21 bp, synthetic construct
  misc_feature 1..21: note = amorce forward COL8A1
  source 1..21: mol_type = other DNA
ccaactcacccttgaagtcat

SEQ ID NO: 8 - DNA, 21 bp, synthetic construct
  misc_feature 1..21: note = amorce reverse COL8A1
  source 1..21: mol_type = other DNA
ggctggtttctgtctcttcag

SEQ ID NO: 9 - DNA, 24 bp, synthetic construct
  misc_feature 1..24: note = amorce forward DDIT3
  source 1..24: mol_type = other DNA
atggcagctgagtcattgcctttc

SEQ ID NO: 10 - DNA, 24 bp, synthetic construct
  misc_feature 1..24: note = amorce reverse DDIT3
  source 1..24: mol_type = other DNA
agaagcagggtcaagagtggtgaa

SEQ ID NO: 11 - DNA, 19 bp, synthetic construct
  misc_feature 1..19: note = amorce forward HSPA5
  source 1..19: mol_type = other DNA
cgaggaggagacaagaagg

SEQ ID NO: 12 - DNA, 20 bp, synthetic construct
  misc_feature 1..20: note = amorce reverse HSPA5
  source 1..20: mol_type = other DNA
caccttgaacggcaagaact

SEQ ID NO: 13 - DNA, 20 bp, synthetic construct
  misc_feature 1..20: note = amorce forward MMP2
  source 1..20: mol_type = other DNA
gtgaagtatgggaacgccga

SEQ ID NO: 14 - DNA, 20 bp, synthetic construct
  misc_feature 1..20: note = amorce reverse MMP2
  source 1..20: mol_type = other DNA
agaagccgtacttgccatcc

SEQ ID NO: 15 - DNA, 20 bp, synthetic construct
  misc_feature 1..20: note = amorce forward MMP14
  source 1..20: mol_type = other DNA
tccagcaactttatgggggt

SEQ ID NO: 16 - DNA, 20 bp, synthetic construct
  misc_feature 1..20: note = amorce reverse MMP14
  source 1..20: mol_type = other DNA
ttcccgtcacagatgttggg

SEQ ID NO: 17 - DNA, 20 bp, synthetic construct
  misc_feature 1..20: note = amorce forward SNAI2
  source 1..20: mol_type = other DNA
tggttgcttcaaggacacat

SEQ ID NO: 18 - DNA, 20 bp, synthetic construct
  misc_feature 1..20: note = amorce reverse SNAI2
  source 1..20: mol_type = other DNA
gcaaatgctctgttgcagtg

SEQ ID NO: 19 - DNA, 20 bp, synthetic construct
  misc_feature 1..20: note = amorce forward sXBP1
  source 1..20: mol_type = other DNA
ctgagtccgaatcaggtgca

SEQ ID NO: 20 - DNA, 21 bp, synthetic construct
  misc_feature 1..21: note = amorce reverse sXBP1
  source 1..21: mol_type = other DNA
atccatggggagatgttctgg

SEQ ID NO: 21 - DNA, 22 bp, synthetic construct
  misc_feature 1..22: note = amorce forward ZO1
  source 1..22: mol_type = other DNA
ggtcagagccttctgatcattc

SEQ ID NO: 22 - DNA, 21 bp, synthetic construct
  misc_feature 1..21: note = amorce reverse ZO1
  source 1..21: mol_type = other DNA
catctctactccggagactgc